European Patent Application EP 4 122 498 A1, published January 25, 2023. Title: COMPOSITION FOR DELIVERY OF GENETIC MATERIAL. Applicant: ISIS INNOVATION LIMITED. The sequence listing filed with the application follows.

SEQUENCE LISTING (24 sequences)

SEQ ID NO: 1 - protein, 415 aa, Mus musculus
MCLSPVKGAKLILIFLFLGAVQSNALIVNLTDSKGTCLYAEWEMNFTITYETTNQTNKTITIAVPDKATHDGSSCGDDRNSAKIMIQFGFAVSWAVNFTKEASHYSIHDIVLSYNTSDSTVFPGAVAKGVHTVKNPENFKVPLDVIFKCNSVLTYNLTPVVQKYWGIHLQAFVQNGTVSKNEQVCEEDQTPTTVAPIIHTTAPSTTTTLTPTSTPTPTPTPTPTVGNYSIRNGNTTCLLATMGLQLNITEEKVPFIFNINPATTNFTGSCQPQSAQLRLNNSQIKYLDFIFAVKNEKRFYLKEVNVYMYLANGSAFNISNKNLSFWDAPLGSSYMCNKEQVLSVSRAFQINTFNLKVQPFNVTKGQYSTAQECSLDDDTILIPIIVGAGLSGLIIVIVIAYLIGRRKTYAGYQTL

SEQ ID NO: 2 - DNA, 1248 bp, Mus musculus
atgtgcctctctccggttaaaggcgcaaagctcatcctgatctttctgttcctaggagccgttcagtccaatgcattgatagttaatttgacagattcaaagggtacttgcctttatgcagaatgggagatgaatttcacaataacatatgaaactacaaaccaaaccaataaaactataaccattgcagtacctgacaaggcgacacacgatggaagcagttgtggggatgaccggaatagtgccaaaataatgatacaatttggattcgctgtctcttgggctgtgaattttaccaaggaagcatctcattattcaattcatgacatcgtgctttcctacaacactagtgatagcacagtatttcctggtgctgtagctaaaggagttcatactgttaaaaatcctgagaatttcaaagttccattggatgtcatctttaagtgcaatagtgttttaacttacaacctgactcctgtcgttcagaaatattggggtattcacctgcaagcttttgtccaaaatggtacagtgagtaaaaatgaacaagtgtgtgaagaagaccaaactcccaccactgtggcacccatcattcacaccactgccccgtcgactacaactacactcactccaacttcaacacccactccaactccaactccaactccaaccgttggaaactacagcattagaaatggcaatactacctgtctgctggctaccatggggctgcagctgaacatcactgaggagaaggtgcctttcatttttaacatcaaccctgccacaaccaacttcaccggcagctgtcaacctcaaagtgctcaacttaggctgaacaacagccaaattaagtatcttgactttatctttgctgtgaaaaatgaaaaacggttctatctgaaggaagtgaatgtctacatgtatttggctaatggctcagctttcaacatttccaacaagaaccttagcttctgggatgcccctctgggaagttcttatatgtgcaacaaagagcaggtgctttctgtgtctagagcgtttcagatcaacacctttaacctaaaggtgcaaccttttaatgtgacaaaaggacagtattctacagcccaggagtgttcgctggatgatgacaccattctaataccaattatagttggtgctggtctttcaggcttgattatcgttatagtgattgcttacctaattggcagaagaaagacctatgctggatatcagactctgtaa

SEQ ID NO: 3 - protein, 40 aa, Artificial Sequence
  Fragment of modified amino acid sequence of murine Lamp 2 isoform 2: N-terminal to peptide tag
MCLSPVKGAKLILIFLFLGAVQSNALIVNLTDSKGTCLYA

SEQ ID NO: 4 - protein, 378 aa, Artificial Sequence
  Fragment of modified amino acid sequence of murine Lamp 2 isoform 2: C-terminal to peptide tag
GGAEWEMNFTITYETTNQTNKTITIAVPDKATHDGSSCGDDRNSAKIMIQFGFAVSWAVNFTKEASHYSIHDIVLSYNTSDSTVFPGAVAKGVHTVKNPENFKVPLDVIFKCNSVLTYNLTPVVQKYWGIHLQAFVQNGTVSKNEQVCEEDQTPTTVAPIIHTTAPSTTTTLTPTSTPTPTPTPTPTVGNYSIRNGNTTCLLATMGLQLNITEEKVPFIFNINPATTNFTGSCQPQSAQLRLNNSQIKYLDFIFAVKNEKRFYLKEVNVYMYLANGSAFNISNKNLSFWDAPLGSSYMCNKEQVLSVSRAFQINTFNLKVQPFNVTKGQYSTAQECSLDDDTILIPIIVGAGLSGLIIVIVIAYLIGRRKTYAGYQTL

SEQ ID NO: 5 - DNA, 1270 bp, Artificial Sequence
  Modified nucleotide sequence of murine Lamp 2 isoform 2
atgtgcctctctccggttaaaggcgcaaagctcatcctgatctttctgttcctaggagccgttcagtccaatgcattgatagttaatttgacagattcaaagggtacttgcctttatgctcgaggtcacatccggaggtgcagaatgggagatgaatttcacaataacatatgaaactacaaaccaaaccaataaaactataaccattgcagtacctgacaaggcgacacacgatggaagcagttgtggggatgaccggaatagtgccaaaataatgatacaatttggattcgctgtctcttgggctgtgaattttaccaaggaagcatctcattattcaattcatgacatcgtgctttcctacaacactagtgatagcacagtatttcctggtgctgtagctaaaggagttcatactgttaaaaatcctgagaatttcaaagttccattggatgtcatctttaagtgcaatagtgttttaacttacaacctgactcctgtcgttcagaaatattggggtattcacctgcaagcttttgtccaaaatggtacagtgagtaaaaatgaacaagtgtgtgaagaagaccaaactcccaccactgtggcacccatcattcacaccactgccccgtcgactacaactacactcactccaacttcaacacccactccaactccaactccaactccaaccgttggaaactacagcattagaaatggcaatactacctgtctgctggctaccatggggctgcagctgaacatcactgaggagaaggtgcctttcatttttaacatcaaccctgccacaaccaacttcaccggcagctgtcaacctcaaagtgctcaacttaggctgaacaacagccaaattaagtatcttgactttatctttgctgtgaaaaatgaaaaacggttctatctgaaggaagtgaatgtctacatgtatttggctaatggctcagctttcaacatttccaacaagaaccttagcttctgggatgcccctctgggaagttcttatatgtgcaacaaagagcaggtgctttctgtgtctagagcgtttcagatcaacacctttaacctaaaggtgcaaccttttaatgtgacaaaaggacagtattctacagcccaggagtgttcgctggatgatgacaccattctaataccaattatagttggtgctggtctttcaggcttgattatcgttatagtgattgcttacctaattggcagaagaaagacctatgctggatatcagactctgtaa

SEQ ID NO: 6 - protein, 29 aa, Artificial Sequence
  neuron-specific rabies viral glycoprotein (RVG)
YTIWMPENPRPGTPCDIFTNSRGKRASNG

SEQ ID NO: 7 - DNA, 92 bp, Artificial Sequence
  RVG forward primer
tcgatacaccatttggatgcccgagaatccgagaccagggacaccttgtgacatttttaccaatagcagagggaagagagcatccaacgggt

SEQ ID NO: 8 - DNA, 92 bp, Artificial Sequence
  RVG reverse primer
ccggacccgttggatgctctcttccctctgctattggtaaaaatgtcacaaggtgtccctggtctcggattctcgggcatccaaatggtgta

SEQ ID NO: 9 - protein, 7 aa, Artificial Sequence
  muscle-specific peptide (MSP) identified by in vivo phage display
ASSLNIA

SEQ ID NO: 10 - DNA, 26 bp, Artificial Sequence
  MSP forward primer
tcgagccagcagcctgaacatcgcct

SEQ ID NO: 11 - DNA, 26 bp, Artificial Sequence
  MSP reverse primer
ccggaggcgatgttcaggctgctggc

SEQ ID NO: 12 - protein, 8 aa, Artificial Sequence
  FLAG
DYKDDDDK

SEQ ID NO: 13 - DNA, 29 bp, Artificial Sequence
  FLAG forward primer
tcgagattacaaggatgacgatgacaagt

SEQ ID NO: 14 - DNA, 29 bp, Artificial Sequence
  FLAG reverse primer
ccggacttgtcatcgtcatccttgtaatc

SEQ ID NO: 15 - DNA, 23 bp, Artificial Sequence
  Cyclophilin-B human forward primer
aaagtcaccgtcaaggtgtattt

SEQ ID NO: 16 - DNA, 22 bp, Artificial Sequence
  Cyclophilin-B human reverse primer
tcaccgtagatgctctttcctc

SEQ ID NO: 17 - DNA, 20 bp, Artificial Sequence
  GAPDH human forward primer
aaggtgaaggtcggagtcaa

SEQ ID NO: 18 - DNA, 20 bp, Artificial Sequence
  GAPDH human reverse primer
gaagatggtgatgggatttc

SEQ ID NO: 19 - DNA, 21 bp, Artificial Sequence
  GAPDH mouse forward primer
caatgtgtccgtcgtggatct

SEQ ID NO: 20 - skipped
  GAPDH mouse reverse primer

SEQ ID NO: 21 - DNA, 19 bp, Artificial Sequence
  eGFP forward primer
tcttcaagtccgccatgcc

SEQ ID NO: 22 - DNA, 19 bp, Artificial Sequence
  eGFP reverse primer
tgtcgccctcgaacttcac

SEQ ID NO: 23 - DNA, 20 bp, Artificial Sequence
  18S forward primer
gtaacccgttgaaccccatt

SEQ ID NO: 24 - DNA, 20 bp, Artificial Sequence
  18S reverse primer
ccatccaatcggtagtagcg